European Patent Specification EP 3 784 792 B9, published October 4, 2023. Title: Enzymatic method for preparation of GDP-fucose. Applicant: Max-Planck-Gesellschaft zur Foerderung der Wissenschaften e.V. The sequence listing filed with the application follows.

SEQUENCE LISTING (16 sequences)

SEQ ID NO: 1 - protein, 321 aa, Escherichia coli
  PEPTIDE (1)..(321): Glucokinase
MTKYALVGDVGGTNARLALCDIASGEISQAKTYSGLDYPSLEAVIRVYLEEHKVEVKDGCIAIACPITGDWVAMTNHTWAFSIAEMKKNLGFSHLEIINDFTAVSMAIPMLKKEHLIQFGGAEPVEGKPIAVYGAGTGLGVAHLVHVDKRWVSLPGEGGHVDFAPNSEEEAIILEILRAEIGHVSAERVLSGPGLVNLYRAIVKADNRLPENLKPKDITERALADSCTDCRRALSLFCVIMGRFGGNLALNLGTFGGVFIAGGIVPRFLEFFKASGFRAAFEDKGRFKEYVHDIPVYLIVHDNPGLLGSGAHLRQTLGHIL

SEQ ID NO: 2 - protein, 456 aa, Escherichia coli
  PEPTIDE (1)..(456): Phosphomannomutase
MKKLTCFKAYDIRGKLGEELNEDIAWRIGRAYGEFLKPKTIVLGGDVRLTSETLKLALAKGLQDAGVDVLDIGMSGTEEIYFATFHLGVDGGIEVTASHNPMDYNGMKLVREGARPISGDTGLRDVQRLAEANDFPPVDETKRGRYQQINLRDAYVDHLFGYINVKNLTPLKLVINSGNGAAGPVVDAIEARFKALGAPVELIKVHNTPDGNFPNGIPNPLLPECRDDTRNAVIKHGADMGIAFDGDFDRCFLFDEKGQFIEGYYIVGLLAEAFLEKNPGAKIIHDPRLSWNTVDVVTAAGGTPVMSKTGHAFIKERMRKEDAIYGGEMSAHHYFRDFAYCDSGMIPWLLVAELVCLKDKTLGELVRDRMAAFPASGEINSKLAQPVEAINRVEQHFSREALAVDRTDGISMTFADWRFNLRTSNTEPVVRLNVESRGDVPLMEARTRTLLTLLNE

SEQ ID NO: 3 - protein, 359 aa, Bifidobacterium longum
  PEPTIDE (1)..(359): N-acetylhexosamine-1-kinase
MTESNEDLFGIASHFALEGAVTGIEPYGDGHINTTYLVTTDGPRYILQQMNTSIFPDTVNLMRNVELVTSTLKAQGKETLDIVPTTSGATWAEIDGGAWRVYKFIEHTVSYNLVPNPDVFREAGSAFGDFQNFLSEFDASQLTETIAHFHDTPHRFEDFKAALAADKLGRAAACQPEIDFYLSHADQYAVVMDGLRDGSIPLRVTHNDTKLNNILMDATTGKARAIIDLDTIMPGSMLFDFGDSIRFGASTALEDEKDLSKVHFSTELFRAYTEGFVGELRGSITAREAELLPFSGNLLTMECGMRFLADYLEGDIYFATKYPEHNLVRTRTQIKLVQEMEQKASETRAIVADIMEAAR

SEQ ID NO: 4 - protein, 478 aa, Escherichia coli
  PEPTIDE (1)..(478): Mannose-1-phosphate guanylyltransferase
MAQSKLYPVVMAGGSGSRLWPLSRVLYPKQFLCLKGDLTMLQTTICRLNGVECESPVVICNEQHRFIVAEQLRQLNKLTENIILEPAGRNTAPAIALAALAAKRHSPESDPLMLVLAADHVIADEDAFRAAVRNAMPYAEAGKLVTFGIVPDLPETGYGYIRRGEVSAGEQDMVAFEVAQFVEKPNLETAQAYVASGEYYWNSGMFLFRAGRYLEELKKYRPDILDACEKAMSAVDPDLNFIRVDEEAFLACPEESVDYAVMERTADAVVVPMDAGWSDVGSWSSLWEISAHTAEGNVCHGDVINHKTENSYVYAESGLVTTVGVKDLVVVQTKDAVLIADRNAVQDVKKVVEQIKADGRHEHRVHREVYRPWGKYDSIDAGDRYQVKRITVKPGEGLSVQMHHHRAEHWVVVAGTAKVTIDGDIKLLGENESIYIPLGATHCLENPGKIPLDLIEVRSGSYLEEDDVVRFADRYGRV

SEQ ID NO: 5 - protein, 373 aa, Escherichia coli [sequence omitted]

SEQ ID NO: 6 - protein, 321 aa, Escherichia coli
  PEPTIDE (1)..(321): GDP-L-fucose synthase
MSKQRVFIAGHRGMVGSAIKRQLEQRGDVELVLRTRDELNLLDSRAVHDFFASESIDQVYLAAAKVGGIVANNTYPADFIYQNMMIESNIIHAAHQNDVNKLLFLGSSCIYPKLAKQPMAESELLQGTLEPTNEPYAIAKIAGIKLCESYNRQYGRDYRSVMPTNLYGPHDNFHPSNSHVIPALLRRFHEATAQNAPDVVVWGSGTPMREFLHVDDMAAASIHVMELAHEVWLENTQPMLSHINVGTGVDCTIRELAQTIAKVVDYKGRVVFDASKPDGTPRKLLDVTRLHQLGWYHEISLEAGLASTYQWFLENRDRFRG

SEQ ID NO: 7 - protein, 949 aa, Bacteroides fragilis
  PEPTIDE (1)..(949): L-fucokinase
MQKLLSLPSNLVQSFHELERVNRTDWFCTSDPVGKKLGSGGGTSWLLEECYNEYSDGATFGEWLEKEKRILLHAGGQSRRLPGYAPSGKILTPVPVFRWERGQHLGQNLLSLQLPLYEKIMSLAPDKLHTLIASGDVYIRSEKPLQSIPEADVVCYGLWVDPSLATHHGVFASDRKHPEQLDFMLQKPSLAELESLSKTHLFLMDIGIWLLSDRAVEILMKRSHKESSEELKYYDLYSDFGLALGTHPRIEDEEVNTLSVAILPLPGGEFYHYGTSKELISSTLSVQNKVYDQRRIMHRKVKPNPAMFVQNAVVRIPLCAENADLWIENSHIGPKWKIASRHIITGVPENDWSLAVPAGVCVDVVPMGDKGFVARPYGLDDVFKGDLRDSKTTLTGIPFGEWMSKRGLSYTDLKGRTDDLQAVSVFPMVNSVEELGLVLRWMLSEPELEEGKNIWLRSEHFSADEISAGANLKRLYAQREEFRKGNWKALAVNHEKSVFYQLDLADAAEDFVRLGLDMPELLPEDALQMSRIHNRMLRARILKLDGKDYRPEEQAAFDLLRDGLLDGISNRKSTPKLDVYSDQIVWGRSPVRIDMAGGWTDTPPYSLYSGGNVVNLAIELNGQPPLQVYVKPCKDFHIVLRSIDMGAMEIVSTFDELQDYKKIGSPFSIPKAALSLAGFAPAFSAVSYASLEEQLKDFGAGIEVTLLAAIPAGSGLGTSSILASTVLGAINDFCGLAWDKNEICQRTLVLEQLLTTGGGWQDQYGGVLQGVKLLQTEAGFAQSPLVRWLPDHLFTHPEYKDCHLLYYTGITRTAKGILAEIVSSMFLNSSLHLNLLSEMKAHALDMNEAIQRGSFVEFGRLVGKTWEQNKALDSGTNPPAVEAIIDLIKDYTLGYKLPGAGGGGYLYMVAKDPQAAVRIRKILTENAPNPRARFVEMTLSDKGFQVSRS

SEQ ID NO: 8 - protein, 303 aa, Exiguobacterium acetylicum
  PEPTIDE (1)..(303): Guanosine kinase
MNKIAVIGKVFVDIKGTSFAPLHKDAKNVGDITFSNGGTGRNVAQNLAVLGNEVRFISTVTNDQIGVGVLDELKSYGANVDHVEMLEDHGMGMWLAVMDNEGDLQTSISKQPDAKLLEEAILRQSIYALDGVDAVAIDLDLSVTVLERLIHLCRKMELPLFGVCGHLSVIERNRHLLQGFTGFICSREEAEILSDLSIVTVEDAIHVANELAKKGAPFTVVTMSELGAVYVDRRTATSGHVGTKKVKVVDSTGAGDSFFSAVLSELTQEKSAEEALKLGMKVAAEVIASTENGLVPEMLDALQ

SEQ ID NO: 9 - protein, 496 aa, Pseudomonas aeruginosa
  PEPTIDE (1)..(496): 2-domain polyphosphate kinase 2
MFESAEVGHSIDKDTYEKAVIELREALLEAQFELKQQARFPVIILINGIEGAGKGETVKLLNEWMDPRLIEVQSFLRPSDEELERPPQWRFWRRLPPKGRTGIFFGNWYSQMLYARVEGHIKEAKLDQAIDAAERFERMLCDEGALLFKFWFHLSKKQLKERLKALEKDPQHSWKLSPLDWKQSEVYDRFVHYGERVLRRTSRDYAPWYVVEGADERYRALTVGRILLEGLQAALATKERAKRQPHAAPLVSSLDNRGLLDSLDLGQYLDKDAYKEQLAAEQARLAGLIRDKRFRQHSLVAVFEGNDAAGKGGAIRRVTDALDPRQYHIVPIAAPTEEERAQPYLWRFWRHIPARRQFTIFDRSWYGRVLVERIEGFCAPADWLRAYGEINDFEEQLSEYGIIVVKFWLAIDKQTQMERFKEREKTPYKRYKITEEDWRNRDKWDQYVDAVGDMVDRTSTEIAPWTLVEANDKRFARVKVLRTINDAIEAAYKKDK

SEQ ID NO: 10 - protein, 177 aa, Pasteurella multocida
  PEPTIDE (1)..(177): inorganic pyrophosphatase
MGLETVPAGKALPDDIYVVIEIPANSDPIKYEVDKESGALFVDRFMATAMFYPANYGYVNNTLSLDGDPVDVLVPTPYPLQPGSVIRCRPVGVLKMTDEAGSDAKVVAVPHSKLTKEYDHIKDVNDLPALLKAQIQHFFESYKALEAGKWVKVDGWEGVDAARQEILDSFERAKKLE

SEQ ID NO: 11 - protein, 198 aa, Sus scrofa
  PEPTIDE (1)..(198): Guanylate kinase
MGSPRPVVLSGPSGAGKSTLLKKLLQEHSSIFGFSVSHTTRDPRPGEENGKDYYFVTREVMQRDIAAGDFIEHAEFSGNLYGTSKAAVRAVQAMNRICVLDVDLQGVRNIKKTDLQPIYIFVQPPSLDVLEQRLRQRNTETEESLAKRLAAAKADMESSKEPGLFDLIIINDSLDKAYWALKEALSEEIKKAQATGHS

SEQ ID NO: 12 - protein, 558 aa, Bos taurus
  PEPTIDE (1)..(558): Glutamate dehydrogenase 1 (GLDH)
MYRYLGEALLLSRAGPAALGSASADSAALLGWARGQPAAAPQPGLVPPARRHYSEAAADREDDPNFFKMVEGFFDRGASIVEDKLVEDLKTRETEEQKRNRVRSILRIIKPCNHVLSLSFPIRRDDGSWEVIEGYRAQHSQHRTPCKGGIRYSTDVSVDEVKALASLMTYKCAVVDVPFGGAKAGVKINPKNYTDNELEKITRRFTMELAKKGFIGPGVDVPAPDMSTGEREMSWIADTYASTIGHYDINAHACVTGKPISQGGIHGRISATGRGVFHGIENFINEASYMSILGMTPGFGDKTFVVQGFGNVGLHSMRYLHRFGAKCITVGESDGSIWNPDGIDPKELEDFKLQHGTILGFPKAKIYEGSILEVDCDILIPAASEKQLTKSNAPRVKAKIIAEGANGPTTPEADKIFLERNIMVIPDLYLNAGGVTVSYFEWLNNLNHVSYGRLTFKYERDSNYHLLMSVQESLERKFGKHGGTIPIVPTAEFQDRISGASEKDIVHSGLAYTMERSARQIMRTAMKYNLGLDLRTAAYVNAIEKVFRVYNEAGVTFT

SEQ ID NO: 13 - protein, 486 aa, Leuconostoc mesenteroides
  PEPTIDE (1)..(486): Glucose-6-phosphate 1-dehydrogenase (G6PDH)
MVSEIKTLVTFFGGTGDLAKRKLYPSVFNLYKKGYLQEHFAIVGTARQQLSDEEFKQLVRDSIKDFTEDQAQAEAFIAHFSYRAHDVTDAASYGILKSAIEEAATKFDIDGNRIFYMSVAPRFFGTIAKYLKSEGLLADTGYNRLMIEKPFGTSYATAEELQSDLENAFDDDQLFRIDHYLGKEMVQNIAALRFGNPIFDAAWNKDYIKNVQVTLSEVLGVEERAGYYDTTGALLDMIQNHTMQIVGWLAMEKPESFNDKDIRAAKNAAFNALKIYNEEEVNKYFVRAQYGAGDTADYKPYLEEADVPADSKNNTFIAGELQFDLPRWEGVPFYVRSGKRLAAKQTRVDIVFKAGTFNFGSEQEAQESVLSIIIDPKGAIELKLNAKSVEDAFNTRTINLDWAVSDEDKKNTPEPYERMIHDTMNGDGSNFADWNGVSIAWKFVDAITAVYDADKAPLETYKSGSMGPEASDKLLAENGDAWVFKG

SEQ ID NO: 14 - protein, 301 aa, Ruegeria pomerovi
  PEPTIDE (1)..(301): phosphotransferase 3 (PPK3)
MNRNGSTKDPRRMTGAATGEISRYFNDKAPKDIRRAIEKADKDDILSTTYPYDAEMTAKDYRAQMEALQIELVKLQAWIKQSGARVALLFEGRDAAGKGGTIKRFRENLNPRGARVVALSKPTEAERSQWYFQRYIQHLPSAGELVFYDRSWYNRGVVEHVFGWCDEEQRERFFRQVMPFEHDLVDDGIHLFKFWLNVGRAEQLRRFHDRERDPLKQWKLSPVDIAGLDKWEAYTTAISQTLTRSHSDRAPWTVIRSDDKKRARLAAIRTVLSGIDYDNKDRAAVGQPDAAICGGPDIWDA

SEQ ID NO: 15 - protein, 359 aa, Picrophilus torridus
  PEPTIDE (1)..(359): Glucose/galactose 1-dehydrogenase (GDH)
MVRAIITNAPNGGVKIENVNINEPEHYEVKLRPVYTGLCGTDRGEVLGNLSFAYNEPGYNYLVLGHEAICQVIEASENPYKIKPGDYVVPVVRRPGKCVNCRIGREDDCSDGDKHEAGITGLHGFMRDYFYDEAKNLVKINDKNMVKVAVLTEPTKNVMKAFEVFDTVSKRSIFQGDDSTNLTKNCLIIGTGSEAFLYAFMAREYRFNVFMTNRHPVGEEKLSIISRINADFYDYTREDPLKGIDLLIDTSGDPGTIFRFVRKMNYNGVVILFGTNGRAPATSIDGEDIDYIIERNISLVGSVDGAKRHYLRAVEYLEKWNYSEGSVINRLITGVFEPEDVSIFTKKPENEIKSVIKWS

SEQ ID NO: 16 - protein, 462 aa, Helicobacter pylori
  PEPTIDE (1)..(462): alpha-1,3/4-fucosyltransferase (3/4FT)
MFQPLLDAFIDSTHLDETTHKPPLNVALANWWPLKNSEKKGFRDFILHFILKQRYKIILHSNPNEPSDLVFGNPLEQARKILSYQNTKRVFYTGENEVPNFNLFDYAIGFDELDFNDRYLRMPLYYAYLHYKAMLVNDTTSPYKLKALYTLKKPSHKFKENHPNLCALIHNESDPWKRGFASFVASNPNAPIRNAFYDALNAIEPVASGGSVKNTLGYKVKNKNEFLSQYKFNLCFENSQGYGYVTEKILDAYFSHTIPIYWGSPSVAKDFNPKSFVNVHDFNNFDEAIDYIRYLHAHQNAYLDMLYENPLNTIDGKAGFYQDLSFEKILDFFKNILENDTIYHCNDAHYSALHRDLNEPLVSVDDLRRDHDDLRVNYDDLRVNYDDLRVNYDDLRVNYDDLRVNYDDLRRDHDDLRRDHERLLSKATPLLELSQNTSFKIYRKAYQKSLPLLRAIRRWVRK